European Patent Application EP 4 435 002 A1, published September 25, 2024. Title: 经修饰的蛋白或多肽. Applicant: 江苏恒瑞医药股份有限公司. Application CN. The sequence listing filed with the application follows.

SEQUENCE LISTING (197 sequences)

SEQ ID NO: 1 - protein, 130 aa, synthetic construct
  source 1..130: note = P2-1
HHHHHHGGGGSEVQLLESGGGLVQPGGSLRLSCAASGFTFAHETMVWVRQAPGKGLEWVSHIPPDGQDPFYADSVKGRFTISRDNSKNTLYLQMNSLRAEDTAVYHCALLPKRGPWFDYWGQGTLVTVSS

SEQ ID NO: 2 - protein, 131 aa, synthetic construct
  source 1..131: note = P2-2
HHHHHHGGGGSEVQLLESGGGLVQPGGSLRLSCAASGFTFAHETMVWVRQAPGKGLEWVSHIPPDGQDPFYADSVKGRFTISRDNSKNTLYLQMNSLRAEDTAVYHCALLPKRGPWFDYWGQGTLVTVSSA

SEQ ID NO: 3 - protein, 449 aa, synthetic construct
  source 1..449: note = heavy chain of IgG1
QVQLKQSGPGLVQPSQSLSITCTVSGFSLTNYGVHWVRQSPGKGLEWLGVIWSGGNTDYNTPFTSRLSINKDNSKSQVFFKMNSLQSNDTAIYYCARALTYYDYEFAYWGQGTLVTVSAASTKGPSVFPLAPSSKSTSGGTAALGCLVKDYFPEPVTVSWNSGALTSGVHTFPAVLQSSGLYSLSSVVTVPSSSLGTQTYICNVNHKPSNTKVDKKVEPKSCDKTHTCPPCPAPELLGGPSVFLFPPKPKDTLMISRTPEVTCVVVDVSHEDPEVKFNWYVDGVEVHNAKTKPREEQYNSTYRVVSVLTVLHQDWLNGKEYKCKVSNKALPAPIEKTISKAKGQPREPQVYTLPPSRDELTKNQVSLTCLVKGFYPSDIAVEWESNGQPENNYKTTPPVLDSDGSFFLYSKLTVDKSRWQQGNVFSCSVMHEALHNHYTQKSLSLSPGK

SEQ ID NO: 4 - protein, 214 aa, synthetic construct
  source 1..214: note = light chain of IgG1
DILLTQSPVILSVSPGERVSFSCRASQSIGTNIHWYQQRTNGSPRLLIKYASESISGIPSRFSGSGSGTDFTLSINSVESEDIADYYCQQNNNWPTTFGAGTKLELKRTVAAPSVFIFPPSDEQLKSGTASVVCLLNNFYPREAKVQWKVDNALQSGNSQESVTEQDSKDSTYSLSSTLTLSKADYEKHKVYACEVTHQGLSSPVTKSFNRGEC

SEQ ID NO: 5 - protein, 163 aa, synthetic construct
  source 1..163: note = 4-1BB
LQDPCSNCPAGTFCDNNRNQICSPCPPNSFSSAGGQRTCDICRQCKGVFRTRKECSSTSNAECDCTPGFHCLGAGCSMCEQDCKQGQELTKKGCKDCCFGTFNDQKRGICRPWTNCSLDGKSVLVNGTKERDVVCGPSPADLSPGASSVTPPAPAREPGHSPQ

SEQ ID NO: 6 - protein, 124 aa, synthetic construct
  source 1..124: note = C5
QVQLVESGGGLVQPGGSLRLSCSASGFTFSSYAMSWVRQAPGKGLEWVSDINSGGESTFYEDSVKGRFTISRDNAKNTLYLQMNSLKPEDTAVYYCAKHPLTFTIATMNDYDYWGQGTQVTVSS

SEQ ID NO: 7 - protein, 5 aa, synthetic construct
  source 1..5: note = CDR1
SYAMS

SEQ ID NO: 8 - protein, 17 aa, synthetic construct
  source 1..17: note = CDR2
DINSGGESTFYEDSVKG

SEQ ID NO: 9 - protein, 15 aa, synthetic construct
  source 1..15: note = CDR3
HPLTFTIATMNDYDY

SEQ ID NO: 10 - protein, 232 aa, synthetic construct
  source 1..232: note = IgG1-Fc varient
EPKSADKTHTCPPCPAPELLGGPSVFLFPPKPKDTLMISRTPEVTCVVVDVEHEDPEVKFNWYVDGVEVHNAKTKPREEQYNSTYRVVSVLTVLHQDWLNGKEYKCKVSNKAFPAPIEKTISKAKGQPREPQVYTLPPSREEMTKNQVSLTCLVKGFYPSDIAVEWESNGQPENNYKTTPPVLDSDGSFFLYSKLTVDKSRWQQGNVFSCSVMHEALHNHYTQKSLSLSPGK

SEQ ID NO: 11 - protein, 232 aa, synthetic construct
  source 1..232: note = IgG1-Fc varient
EPKSADKTHTCPPCPAPEAAGGPSVFLFPPKPKDTLMISRTPEVTCVVVDVSHEDPEVKFNWYVDGVEVHNAKTKPREEQYASTYRVVSVLTVLHQDWLNGKEYKCKVSNKALPAPIEKTISKAKGQPREPQVYTLPPSREEMTKNQVSLTCLVKGFYPSDIAVEWESNGQPENNYKTTPPVLDSDGSFFLYSKLTVDKSRWQQGNVFSCSVMHEALHNHYTQKSLSLSPGK

SEQ ID NO: 12 - protein, 229 aa, synthetic construct
  source 1..229: note = IgG4-Fc varient
ESKYGPPCPPCPAPEFLGGPSVFLFPPKPKDTLMISRTPEVTCVVVDVSQEDPEVQFNWYVDGVEVHNAKTKPREEQFNSTYRVVSVLTVLHQDWLNGKEYKCKVSNKGLPSSIEKTISKAKGQPREPQVYTLPPSQEEMTKNQVSLTCLVKGFYPSDIAVEWESNGQPENNYKTTPPVLDSDGSFFLYSRLTVDKSRWQEGNVFSCSVMHEALHNHYTQKSLSLSLGK

SEQ ID NO: 13 - protein, 227 aa, synthetic construct
  source 1..227: note = IgG1 Fc
DKTHTCPPCPAPELLGGPSVFLFPPKPKDTLMISRTPEVTCVVVDVSHEDPEVKFNWYVDGVEVHNAKTKPREEQYNSTYRVVSVLTVLHQDWLNGKEYKCKVSNKALPAPIEKTISKAKGQPREPQVYTLPPSRDELTKNQVSLTCLVKGFYPSDIAVEWESNGQPENNYKTTPPVLDSDGSFFLYSKLTVDKSRWQQGNVFSCSVMHEALHNHYTQKSLSLSPGK

SEQ ID NO: 14 - protein, 356 aa, synthetic construct
  source 1..356: note = C5-Fc
QVQLVESGGGLVQPGGSLRLSCSASGFTFSSYAMSWVRQAPGKGLEWVSDINSGGESTFYEDSVKGRFTISRDNAKNTLYLQMNSLKPEDTAVYYCAKHPLTFTIATMNDYDYWGQGTQVTVSSEPKSADKTHTCPPCPAPELLGGPSVFLFPPKPKDTLMISRTPEVTCVVVDVEHEDPEVKFNWYVDGVEVHNAKTKPREEQYNSTYRVVSVLTVLHQDWLNGKEYKCKVSNKAFPAPIEKTISKAKGQPREPQVYTLPPSREEMTKNQVSLTCLVKGFYPSDIAVEWESNGQPENNYKTTPPVLDSDGSFFLYSKLTVDKSRWQQGNVFSCSVMHEALHNHYTQKSLSLSPGA

SEQ ID NO: 15 - protein, 124 aa, synthetic construct
  source 1..124: note = C5_V1
QVQLVESGGGLVQPGGSLRLSCSASGFTFSSYAMSWVRQAPGKGLEWVSDINSGGESTFYEDSVKGRFTISRDNAKNTLYLQMNSLRAEDTAVYYCARHPLTFTIATMNDYDYWGQGTLVTVSS

SEQ ID NO: 16 - protein, 124 aa, synthetic construct
  source 1..124: note = C5_V2
QVQLVESGGGLVQPGGSLRLSCSASGFTFSSYAMSWVRQAPGKGLEWVSDINSGGESTFYEDSVKGRFTISRDNAKNTLYLQMNSLRAEDTAVYYCAKHPLTFTIATMNDYDYWGQGTLVTVSS

SEQ ID NO: 17 - protein, 124 aa, synthetic construct
  source 1..124: note = C5_V3
QVQLVESGGGLVQPGGSLRLSCSASGFTFSSYAMSWVRQAPGKGLEWVSDINSGGESTFYEDSVKGRFTISRDNAKNTLYLQMNSLKPEDTAVYYCAKHPLTFTIATMNDYDYWGQGTLVTVSS

SEQ ID NO: 18 - protein, 124 aa, synthetic construct
  source 1..124: note = C5_V2-YTI
QVQLVESGGGLVQPGGSLRLSCSASGFTFSSYAMSWVRQAPGKGLEWVSDINSGGESTFYEDSVKGRFTISRDNAKNTLYLQMNSLRAEDTAVYYCAKHPLTYTIATMNDYDYWGQGTLVTVSS

SEQ ID NO: 19 - protein, 15 aa, synthetic construct
  source 1..15: note = C5_V2-YTI CDR3
HPLTYTIATMNDYDY

SEQ ID NO: 20 - skipped

SEQ ID NO: 21 - protein, 125 aa, synthetic construct
  source 1..125: note = C5_V2-YTI-43
QVQLVESGGGLVQPGGSLRLSCSASGFTFSSYAMSWVRQAPGKGLEWVSDINSGGESTFYEDSVKGRFTISRDNAKNTLYLQMNSLRAEDTAVYYCAKHPLTYTIATMNDYDYWGQGTLVTVSSA

SEQ ID NO: 22 - protein, 124 aa, synthetic construct
  source 1..124: note = C5_V2-YTI-44
QVQLVESGGGLVQPGGSLRLSCSASGFTFSSYAMSWVRQAPGKGLEWVSDINSGGESTFYEDSVKGRFTISRDNAKNTLYLQMNSLRAEDTAVYYCAKHPLTYTIATMNDYDYWGQGTLVTVSA

SEQ ID NO: 23 - protein, 124 aa, synthetic construct
  source 1..124: note = C5_V2-YTI-46
QVQLVESGGGLVQPGGSLRLSCSASGFTFSSYAMSWVRQAPGKGLEWVSDINSGGESTFYEDSVKGRFTISRDNAKNTLYLQMNSLRAEDTAVYYCAKHPLTYTIATMNDYDYWGQGTLVTVSF

SEQ ID NO: 24 - protein, 124 aa, synthetic construct
  source 1..124: note = C5_V2-YTI-47
QVQLVESGGGLVQPGGSLRLSCSASGFTFSSYAMSWVRQAPGKGLEWVSDINSGGESTFYEDSVKGRFTISRDNAKNTLYLQMNSLRAEDTAVYYCAKHPLTYTIATMNDYDYWGQGTLVTVSG

SEQ ID NO: 25 - protein, 124 aa, synthetic construct
  source 1..124: note = C5_V2-YTI-48
QVQLVESGGGLVQPGGSLRLSCSASGFTFSSYAMSWVRQAPGKGLEWVSDINSGGESTFYEDSVKGRFTISRDNAKNTLYLQMNSLRAEDTAVYYCAKHPLTYTIATMNDYDYWGQGTLVTVSL

SEQ ID NO: 26 - protein, 124 aa, synthetic construct
  source 1..124: note = C5_V2-YTI-49
QVQLVESGGGLVQPGGSLRLSCSASGFTFSSYAMSWVRQAPGKGLEWVSDINSGGESTFYEDSVKGRFTISRDNAKNTLYLQMNSLRAEDTAVYYCAKHPLTYTIATMNDYDYWGQGTLVTVSP

SEQ ID NO: 27 - protein, 124 aa, synthetic construct
  source 1..124: note = C5_V2-YTI-50
QVQLVESGGGLVQPGGSLRLSCSASGFTFSSYAMSWVRQAPGKGLEWVSDINSGGESTFYEDSVKGRFTISRDNAKNTLYLQMNSLRAEDTAVYYCAKHPLTYTIATMNDYDYWGQGTLVTVSR

SEQ ID NO: 28 - protein, 124 aa, synthetic construct
  source 1..124: note = C5_V2-YTI-51
QVQLVESGGGLVQPGGSLRLSCSASGFTFSSYAMSWVRQAPGKGLEWVSDINSGGESTFYEDSVKGRFTISRDNAKNTLYLQMNSLRAEDTAVYYCAKHPLTYTIATMNDYDYWGQGTLVTVST

SEQ ID NO: 29 - protein, 124 aa, synthetic construct
  source 1..124: note = C5_V2-YTI-52
QVQLVESGGGLVQPGGSLRLSCSASGFTFSSYAMSWVRQAPGKGLEWVSDINSGGESTFYEDSVKGRFTISRDNAKNTLYLQMNSLRAEDTAVYYCAKHPLTYTIATMNDYDYWGQGTLVTVSV

SEQ ID NO: 30 - protein, 125 aa, synthetic construct
  source 1..125: note = C5_V2-YTI-53
QVQLVESGGGLVQPGGSLRLSCSASGFTFSSYAMSWVRQAPGKGLEWVSDINSGGESTFYEDSVKGRFTISRDNAKNTLYLQMNSLRAEDTAVYYCAKHPLTYTIATMNDYDYWGQGTLVTVSAA

SEQ ID NO: 31 - protein, 124 aa, synthetic construct
  source 1..124: note = C5_V2-YTI-54
QVQLVESGGGLVQPGGSLRLSCSASGFTFSSYAMSWVRQAPGKGLEWVSDINSGGESTFYEDSVKGRFTISRDNAKNTLYLQMNSLRAEDTAVYYCAKHPLTYTIATMNDYDYWGQGTLVTVFP

SEQ ID NO: 32 - protein, 125 aa, synthetic construct
  source 1..125: note = C5_V2-YTI-55
QVQLVESGGGLVQPGGSLRLSCSASGFTFSSYAMSWVRQAPGKGLEWVSDINSGGESTFYEDSVKGRFTISRDNAKNTLYLQMNSLRAEDTAVYYCAKHPLTYTIATMNDYDYWGQGTLVTVFPA

SEQ ID NO: 33 - protein, 124 aa, synthetic construct
  source 1..124: note = C5_V2-YTI-56
QVQLVESGGGLVQPGGSLRLSCSASGFTFSSYAMSWVRQAPGKGLEWVSDINSGGESTFYEDSVKGRFTISRDNAKNTLYLQMNSLRAEDTAVYYCAKHPLTYTIATMNDYDYWGQGTLVTVRP

SEQ ID NO: 34 - protein, 124 aa, synthetic construct
  source 1..124: note = C5_V2-YTI-57
QVQLVESGGGLVQPGGSLRLSCSASGFTFSSYAMSWVRQAPGKGLEWVSDINSGGESTFYEDSVKGRFTISRDNAKNTLYLQMNSLRAEDTAVYYCAKHPLTYTIATMNDYDYWGQGTLVTVRS

SEQ ID NO: 35 - protein, 125 aa, synthetic construct
  source 1..125: note = C5_V2-YTI-58
QVQLVESGGGLVQPGGSLRLSCSASGFTFSSYAMSWVRQAPGKGLEWVSDINSGGESTFYEDSVKGRFTISRDNAKNTLYLQMNSLRAEDTAVYYCAKHPLTYTIATMNDYDYWGQGTLVTVRSA

SEQ ID NO: 36 - protein, 355 aa, synthetic construct
  source 1..355: note = C5_V2-YTI-42
DKTHTCPPCPAPELLGGPSVFLFPPKPKDTLMISRTPEVTCVVVDVSHEDPEVKFNWYVDGVEVHNAKTKPREEQYNSTYRVVSVLTVLHQDWLNGKEYKCKVSNKALPAPIEKTISKAKGQPREPQVYTLPPSRDELTKNQVSLTCLVKGFYPSDIAVEWESNGQPENNYKTTPPVLDSDGSFFLYSKLTVDKSRWQQGNVFSCSVMHEALHNHYTQKSLSLSPGKGGGGQVQLVESGGGLVQPGGSLRLSCSASGFTFSSYAMSWVRQAPGKGLEWVSDINSGGESTFYEDSVKGRFTISRDNAKNTLYLQMNSLRAEDTAVYYCAKHPLTYTIATMNDYDYWGQGTLVTVSS

SEQ ID NO: 37 - protein, 6 aa, synthetic construct
VTVSAA

SEQ ID NO: 38 - protein, 5 aa, synthetic construct
VTVFP

SEQ ID NO: 39 - protein, 6 aa, synthetic construct
VTVFPA

SEQ ID NO: 40 - protein, 5 aa, synthetic construct
VTVRP

SEQ ID NO: 41 - protein, 4 aa, synthetic construct
VTVR

SEQ ID NO: 42 - protein, 5 aa, synthetic construct
VTVRA

SEQ ID NO: 43 - protein, 5 aa, synthetic construct
VTVFS

SEQ ID NO: 44 - protein, 5 aa, synthetic construct
VTVSP

SEQ ID NO: 45 - protein, 5 aa, synthetic construct
VTVRS

SEQ ID NO: 46 - protein, 6 aa, synthetic construct
VTVRSA

SEQ ID NO: 47 - protein, 4 aa, synthetic construct
SAST

SEQ ID NO: 48 - protein, 5 aa, synthetic construct
SASTK

SEQ ID NO: 49 - protein, 6 aa, synthetic construct
SASTKG

SEQ ID NO: 50 - protein, 7 aa, synthetic construct
SASTKGP

SEQ ID NO: 51 - protein, 4 aa, synthetic construct
SATV

SEQ ID NO: 52 - protein, 4 aa, synthetic construct
SAAS

SEQ ID NO: 53 - protein, 5 aa, synthetic construct
SAAST

SEQ ID NO: 54 - protein, 6 aa, synthetic construct
SAASTK

SEQ ID NO: 55 - protein, 7 aa, synthetic construct
SAASTKG

SEQ ID NO: 56 - protein, 8 aa, synthetic construct
SAASTKGP

SEQ ID NO: 57 - protein, 4 aa, synthetic construct
FSAS

SEQ ID NO: 58 - protein, 5 aa, synthetic construct
FSAST

SEQ ID NO: 59 - protein, 6 aa, synthetic construct
FSASTK

SEQ ID NO: 60 - protein, 7 aa, synthetic construct
FSASTKG

SEQ ID NO: 61 - protein, 8 aa, synthetic construct
FSASTKGP

SEQ ID NO: 62 - protein, 4 aa, synthetic construct
FSTV

SEQ ID NO: 63 - protein, 4 aa, synthetic construct
FPAS

SEQ ID NO: 64 - protein, 5 aa, synthetic construct
FPAST

SEQ ID NO: 65 - protein, 6 aa, synthetic construct
FPASTK

SEQ ID NO: 66 - protein, 7 aa, synthetic construct
FPASTKG

SEQ ID NO: 67 - protein, 8 aa, synthetic construct
FPASTKGP

SEQ ID NO: 68 - protein, 4 aa, synthetic construct
RPAA

SEQ ID NO: 69 - protein, 5 aa, synthetic construct
RPAST

SEQ ID NO: 70 - protein, 6 aa, synthetic construct
RPASTK

SEQ ID NO: 71 - protein, 7 aa, synthetic construct
RPASTKG

SEQ ID NO: 72 - protein, 8 aa, synthetic construct
RPASTKGP

SEQ ID NO: 73 - protein, 4 aa, synthetic construct
RPTV

SEQ ID NO: 74 - protein, 6 aa, synthetic construct
RPAAST

SEQ ID NO: 75 - protein, 7 aa, synthetic construct
RPAASTK

SEQ ID NO: 76 - protein, 8 aa, synthetic construct
RPAASTKG

SEQ ID NO: 77 - protein, 9 aa, synthetic construct
RPAASTKGP

SEQ ID NO: 78 - protein, 4 aa, synthetic construct
RAST

SEQ ID NO: 79 - protein, 5 aa, synthetic construct
RASTK

SEQ ID NO: 80 - protein, 6 aa, synthetic construct
RASTKG

SEQ ID NO: 81 - protein, 7 aa, synthetic construct
RASTKGP

SEQ ID NO: 82 - protein, 5 aa, synthetic construct
RAAST

SEQ ID NO: 83 - protein, 6 aa, synthetic construct
RAASTK

SEQ ID NO: 84 - protein, 7 aa, synthetic construct
RAASTKG

SEQ ID NO: 85 - protein, 8 aa, synthetic construct
RAASTKGP

SEQ ID NO: 86 - protein, 4 aa, synthetic construct
RATV

SEQ ID NO: 87 - protein, 4 aa, synthetic construct
SAAG

SEQ ID NO: 88 - protein, 5 aa, synthetic construct
SAAGG

SEQ ID NO: 89 - protein, 4 aa, synthetic construct
FPGG

SEQ ID NO: 90 - protein, 4 aa, synthetic construct
FPAG

SEQ ID NO: 91 - protein, 5 aa, synthetic construct
FPAGG

SEQ ID NO: 92 - protein, 4 aa, synthetic construct
RAGG

SEQ ID NO: 93 - protein, 4 aa, synthetic construct
RSAA

SEQ ID NO: 94 - protein, 5 aa, synthetic construct
RSAAA

SEQ ID NO: 95 - protein, 4 aa, synthetic construct
RSAS

SEQ ID NO: 96 - protein, 5 aa, synthetic construct
RSAST

SEQ ID NO: 97 - protein, 6 aa, synthetic construct
RSASTK

SEQ ID NO: 98 - protein, 7 aa, synthetic construct
RSASTKG

SEQ ID NO: 99 - protein, 8 aa, synthetic construct
RSASTKGP

SEQ ID NO: 100 - protein, 4 aa, synthetic construct
RSGG

SEQ ID NO: 101 - protein, 5 aa, synthetic construct
VTVSA

SEQ ID NO: 102 - protein, 6 aa, synthetic construct
VTVSAS

SEQ ID NO: 103 - protein, 7 aa, synthetic construct
VTVSAST

SEQ ID NO: 104 - protein, 8 aa, synthetic construct
VTVSASTK

SEQ ID NO: 105 - protein, 9 aa, synthetic construct
VTVSASTKG

SEQ ID NO: 106 - protein, 10 aa, synthetic construct
VTVSASTKGP

SEQ ID NO: 107 - protein, 6 aa, synthetic construct
VTVSAT

SEQ ID NO: 108 - protein, 7 aa, synthetic construct
VTVSATV

SEQ ID NO: 109 - protein, 7 aa, synthetic construct
VTVSAAS

SEQ ID NO: 110 - protein, 8 aa, synthetic construct
VTVSAAST

SEQ ID NO: 111 - protein, 9 aa, synthetic construct
VTVSAASTK

SEQ ID NO: 112 - protein, 10 aa, synthetic construct
VTVSAASTKG

SEQ ID NO: 113 - protein, 11 aa, synthetic construct
VTVSAASTKGP

SEQ ID NO: 114 - protein, 6 aa, synthetic construct
VTVSAT

SEQ ID NO: 115 - protein, 7 aa, synthetic construct
VTVSATV

SEQ ID NO: 116 - protein, 5 aa, synthetic construct
VTVFS

SEQ ID NO: 117 - protein, 6 aa, synthetic construct
VTVFSA

SEQ ID NO: 118 - protein, 7 aa, synthetic construct
VTVFSAS

SEQ ID NO: 119 - protein, 8 aa, synthetic construct
VTVFSAST

SEQ ID NO: 120 - protein, 9 aa, synthetic construct
VTVFSASTK

SEQ ID NO: 121 - protein, 10 aa, synthetic construct
VTVFSASTKG

SEQ ID NO: 122 - protein, 11 aa, synthetic construct
VTVFSASTKGP

SEQ ID NO: 123 - protein, 6 aa, synthetic construct
VTVFST

SEQ ID NO: 124 - protein, 7 aa, synthetic construct
VTVFSTV

SEQ ID NO: 125 - protein, 7 aa, synthetic construct
VTVFPAS

SEQ ID NO: 126 - protein, 8 aa, synthetic construct
VTVFPAST

SEQ ID NO: 127 - protein, 9 aa, synthetic construct
VTVFPASTK

SEQ ID NO: 128 - protein, 10 aa, synthetic construct
VTVFPASTKG

SEQ ID NO: 129 - protein, 11 aa, synthetic construct
VTVFPASTKGP

SEQ ID NO: 130 - protein, 6 aa, synthetic construct
VTVRPA

SEQ ID NO: 131 - protein, 7 aa, synthetic construct
VTVRPAA

SEQ ID NO: 132 - protein, 8 aa, synthetic construct
VTVRPAST

SEQ ID NO: 133 - protein, 9 aa, synthetic construct
VTVRPASTK

SEQ ID NO: 134 - protein, 10 aa, synthetic construct
VTVRPASTKG

SEQ ID NO: 135 - protein, 11 aa, synthetic construct
VTVRPASTKGP

SEQ ID NO: 136 - protein, 7 aa, synthetic construct
VTVRPAA

SEQ ID NO: 137 - protein, 6 aa, synthetic construct
VTVRPT

SEQ ID NO: 138 - protein, 7 aa, synthetic construct
VTVRPTV

SEQ ID NO: 139 - protein, 9 aa, synthetic construct
VTVRPAAST

SEQ ID NO: 140 - protein, 10 aa, synthetic construct
VTVRPAASTK

SEQ ID NO: 141 - protein, 11 aa, synthetic construct
VTVRPAASTKG

SEQ ID NO: 142 - protein, 12 aa, synthetic construct
VTVRPAASTKGP

SEQ ID NO: 143 - protein, 6 aa, synthetic construct
VTVRAA

SEQ ID NO: 144 - protein, 7 aa, synthetic construct
VTVRAST

SEQ ID NO: 145 - protein, 8 aa, synthetic construct
VTVRASTK

SEQ ID NO: 146 - protein, 9 aa, synthetic construct
VTVRASTKG

SEQ ID NO: 147 - protein, 10 aa, synthetic construct
VTVRASTKGP

SEQ ID NO: 148 - protein, 8 aa, synthetic construct
VTVRAAST

SEQ ID NO: 149 - protein, 9 aa, synthetic construct
VTVRAASTK

SEQ ID NO: 150 - protein, 10 aa, synthetic construct
VTVRAASTKG

SEQ ID NO: 151 - protein, 11 aa, synthetic construct
VTVRAASTKGP

SEQ ID NO: 152 - protein, 6 aa, synthetic construct
VTVRAT

SEQ ID NO: 153 - protein, 7 aa, synthetic construct
VTVRATV

SEQ ID NO: 154 - protein, 7 aa, synthetic construct
VTVSAAG

SEQ ID NO: 155 - protein, 8 aa, synthetic construct
VTVSAAGG

SEQ ID NO: 156 - protein, 6 aa, synthetic construct
VTVFPG

SEQ ID NO: 157 - protein, 7 aa, synthetic construct
VTVFPGG

SEQ ID NO: 158 - protein, 7 aa, synthetic construct
VTVFPAG

SEQ ID NO: 159 - protein, 8 aa, synthetic construct
VTVFPAGG

SEQ ID NO: 160 - protein, 6 aa, synthetic construct
VTVRAG

SEQ ID NO: 161 - protein, 7 aa, synthetic construct
VTVRAGG

SEQ ID NO: 162 - protein, 5 aa, synthetic construct
VTVRS

SEQ ID NO: 163 - protein, 6 aa, synthetic construct
VTVRSA

SEQ ID NO: 164 - protein, 7 aa, synthetic construct
VTVRSAA

SEQ ID NO: 165 - protein, 8 aa, synthetic construct
VTVRSAAA

SEQ ID NO: 166 - protein, 7 aa, synthetic construct
VTVRSAS

SEQ ID NO: 167 - protein, 8 aa, synthetic construct
VTVRSAST

SEQ ID NO: 168 - protein, 9 aa, synthetic construct
VTVRSASTK

SEQ ID NO: 169 - protein, 10 aa, synthetic construct
VTVRSASTKG

SEQ ID NO: 170 - protein, 11 aa, synthetic construct
VTVRSASTKGP

SEQ ID NO: 171 - protein, 6 aa, synthetic construct
VTVRSG

SEQ ID NO: 172 - protein, 7 aa, synthetic construct
VTVRSGG

SEQ ID NO: 173 - protein, 4 aa, synthetic construct
AAAA

SEQ ID NO: 174 - protein, 4 aa, synthetic construct
PAAA

SEQ ID NO: 175 - protein, 4 aa, synthetic construct
ASTK

SEQ ID NO: 176 - protein, 5 aa, synthetic construct
ASTKG

SEQ ID NO: 177 - protein, 6 aa, synthetic construct
ASTKGP

SEQ ID NO: 178 - protein, 4 aa, synthetic construct
PAST

SEQ ID NO: 179 - protein, 5 aa, synthetic construct
PASTK

SEQ ID NO: 180 - protein, 6 aa, synthetic construct
PASTKG

SEQ ID NO: 181 - protein, 7 aa, synthetic construct
PASTKGP

SEQ ID NO: 182 - protein, 4 aa, synthetic construct
SAAA

SEQ ID NO: 183 - protein, 5 aa, synthetic construct
SSAST

SEQ ID NO: 184 - protein, 6 aa, synthetic construct
SSASTK

SEQ ID NO: 185 - protein, 7 aa, synthetic construct
SSASTKG

SEQ ID NO: 186 - protein, 8 aa, synthetic construct
SSASTKGP

SEQ ID NO: 187 - protein, 4 aa, synthetic construct
SRSG

SEQ ID NO: 188 - protein, 5 aa, synthetic construct
SRSGG

SEQ ID NO: 189 - protein, 5 aa, synthetic construct
VTVSS

SEQ ID NO: 190 - protein, 6 aa, synthetic construct
VTVSSA

SEQ ID NO: 191 - protein, 5 aa, synthetic construct
VTVSF

SEQ ID NO: 192 - protein, 5 aa, synthetic construct
VTVSG

SEQ ID NO: 193 - protein, 5 aa, synthetic construct
VTVSL

SEQ ID NO: 194 - protein, 5 aa, synthetic construct
VTVSR

SEQ ID NO: 195 - protein, 5 aa, synthetic construct
VTVST

SEQ ID NO: 196 - protein, 5 aa, synthetic construct
VTVSV

SEQ ID NO: 197 - protein, 4 aa, synthetic construct
GGGG